European Patent Specification EP 3 901 169 B1, published January 28, 2026. Title: T CELL RECEPTORS RECOGNIZING HLA-CW8 RESTRICTED MUTATED KRAS. Applicant: THE UNITED STATES OF AMERICA, AS REPRESENTED BY THE SECRETARY, DEPARTMENT OF HEALTH AND HUMAN SERVICES. The sequence listing filed with the application follows.

SEQUENCE LISTING (33 sequences)

SEQ ID NO: 1 - protein, 189 aa, Homo sapiens [sequence omitted]

SEQ ID NO: 2 - protein, 188 aa, Homo sapiens [sequence omitted]

SEQ ID NO: 3 - protein, 7 aa, Homo sapiens
NIATNDY

SEQ ID NO: 4 - protein, 5 aa, Homo sapiens
GYKTK

SEQ ID NO: 5 - protein, 13 aa, Homo sapiens
LVGDMDQAGTALI

SEQ ID NO: 6 - protein, 5 aa, Homo sapiens
SGHDT

SEQ ID NO: 7 - protein, 6 aa, Homo sapiens
YYEEEE

SEQ ID NO: 8 - protein, 12 aa, Homo sapiens
ASSLGQTNYGYT

SEQ ID NO: 9 - protein, 129 aa, Homo sapiens
MRQVARVIVFLTLSTLSLAKTTQPISMDSYEGQEVNITCSHNNIATNDYITWYQQFPSQGPRFIIQGYKTKVTNEVASLFIPADRKSSTLSLPRVSLSDTAVYYCLVGDMDQAGTALIFGKGTTLSVSS

SEQ ID NO: 10 - protein, 132 aa, Homo sapiens
MGPGLLCWALLCLLGAGLVDAGVTQSPTHLIKTRGQQVTLRCSPKSGHDTVSWYQQALGQGPQFIFQYYEEEERQRGNFPDRFSGHQFPNYSSELNVNALLLGDSALYLCASSLGQTNYGYTFGSGTRLTVV

SEQ ID NO: 11 - protein, 137 aa, Artificial Sequence
  Synthetic
  MISC_FEATURE (48)..(48): X at position 48 is Thr or Cys
  MISC_FEATURE (112)..(112): X at position 112 is Ser, Ala, Val, Leu, Ile, Pro, Phe, Met, or Trp
  MISC_FEATURE (114)..(114): X at position 114 is Met, Ala, Val, Leu, Ile, Pro, Phe, or Trp
  MISC_FEATURE (115)..(115): X at position 115 is Gly, Ala, Val, Leu, Ile, Pro, Phe, Met, or Trp
DIQNPEPAVYQLKDPRSQDSTLCLFTDFDSQINVPKTMESGTFITDKXVLDMKAMDSKSNGAIAWSNQTSFTCQDIFKETNATYPSSDVPCDATLTEKSFETDMNLNFQNLXVXXLRILLLKVAGFNLLMTLRLWSS

SEQ ID NO: 12 - protein, 173 aa, Artificial Sequence
  Synthetic
  MISC_FEATURE (57)..(57): X at position 57 is Ser or Cys
EDLRNVTPPKVSLFEPSKAEIANKQKATLVCLARGFFPDHVELSWWVNGKEVHSGVXTDPQAYKESNYSYCLSSRLRVSATFWHNPRNHFRCQVQFHGLSEEDKWPEGSPKPVTQNISAEAWGRADCGITSASYQQGVLSATILYEILLGKATLYAVLVSTLVVMAMVKRKNS

SEQ ID NO: 13 - protein, 266 aa, Artificial Sequence
  Synthetic
  MISC_FEATURE (177)..(177): X at position 177 is Thr or Cys
  MISC_FEATURE (241)..(241): X at position 241 is Ser, Ala, Val, Leu, Ile, Pro, Phe, Met, or Trp
  MISC_FEATURE (243)..(243): X at position 243 is Met, Ala, Val, Leu, Ile, Pro, Phe, or Trp
  MISC_FEATURE (244)..(244): X at position 244 is Gly, Ala, Val, Leu, Ile, Pro, Phe, Met, or Trp
MRQVARVIVFLTLSTLSLAKTTQPISMDSYEGQEVNITCSHNNIATNDYITWYQQFPSQGPRFIIQGYKTKVTNEVASLFIPADRKSSTLSLPRVSLSDTAVYYCLVGDMDQAGTALIFGKGTTLSVSSDIQNPEPAVYQLKDPRSQDSTLCLFTDFDSQINVPKTMESGTFITDKXVLDMKAMDSKSNGAIAWSNQTSFTCQDIFKETNATYPSSDVPCDATLTEKSFETDMNLNFQNLXVXXLRILLLKVAGFNLLMTLRLWSS

SEQ ID NO: 14 - protein, 305 aa, Artificial Sequence
  Synthetic
  MISC_FEATURE (189)..(189): X at position 189 is Ser or Cys
MGPGLLCWALLCLLGAGLVDAGVTQSPTHLIKTRGQQVTLRCSPKSGHDTVSWYQQALGQGPQFIFQYYEEEERQRGNFPDRFSGHQFPNYSSELNVNALLLGDSALYLCASSLGQTNYGYTFGSGTRLTVVEDLRNVTPPKVSLFEPSKAEIANKQKATLVCLARGFFPDHVELSWWVNGKEVHSGVXTDPQAYKESNYSYCLSSRLRVSATFWHNPRNHFRCQVQFHGLSEEDKWPEGSPKPVTQNISAEAWGRADCGITSASYQQGVLSATILYEILLGKATLYAVLVSTLVVMAMVKRKNS

SEQ ID NO: 15 - protein, 189 aa, Homo sapiens
MTEYKLVVVGADGVGKSALTIQLIQNHFVDEYDPTIEDSYRKQVVIDGETCLLDILDTAGQEEYSAMRDQYMRTGEGFLCVFAINNTKSFEDIHHYREQIKRVKDSEDVPMVLVGNKCDLPSRTVDTKQAQDLARSYGIPFIETSAKTRQRVEDAFYTLVREIRQYRLKKISKEEKTPGCVKIKKCIIM

SEQ ID NO: 16 - protein, 188 aa, Homo sapiens [sequence omitted]

SEQ ID NO: 17 - protein, 9 aa, Homo sapiens
GAGGVGKSA

SEQ ID NO: 18 - protein, 9 aa, Homo sapiens
GADGVGKSA

SEQ ID NO: 19 - protein, 24 aa, Homo sapiens
MTEYKLVVVGAGGVGKSALTIQLI

SEQ ID NO: 20 - protein, 24 aa, Homo sapiens
MTEYKLVVVGADGVGKSALTIQLI

SEQ ID NO: 21 - DNA, 26 bp, Artificial Sequence
  Synthetic
gccacagcactgtgctcttgaagtcc

SEQ ID NO: 22 - DNA, 24 bp, Artificial Sequence
  Synthetic
caggcagtatctggagtcattgag

SEQ ID NO: 23 - protein, 27 aa, Artificial Sequence
  Synthetic
RAKRSGSGATNFSLLKQAGDVEENPGP

SEQ ID NO: 24 - protein, 137 aa, Mus musculus
DIQNPEPAVYQLKDPRSQDSTLCLFTDFDSQINVPKTMESGTFITDKTVLDMKAMDSKSNGAIAWSNQTSFTCQDIFKETNATYPSSDVPCDATLTEKSFETDMNLNFQNLSVMGLRILLLKVAGFNLLMTLRLWSS

SEQ ID NO: 25 - protein, 173 aa, Mus musculus
EDLRNVTPPKVSLFEPSKAEIANKQKATLVCLARGFFPDHVELSWWVNGKEVHSGVSTDPQAYKESNYSYCLSSRLRVSATFWHNPRNHFRCQVQFHGLSEEDKWPEGSPKPVTQNISAEAWGRADCGITSASYQQGVLSATILYEILLGKATLYAVLVSTLVVMAMVKRKNS

SEQ ID NO: 26 - protein, 266 aa, Artificial Sequence
  Synthetic
MRQVARVIVFLTLSTLSLAKTTQPISMDSYEGQEVNITCSHNNIATNDYITWYQQFPSQGPRFIIQGYKTKVTNEVASLFIPADRKSSTLSLPRVSLSDTAVYYCLVGDMDQAGTALIFGKGTTLSVSSDIQNPEPAVYQLKDPRSQDSTLCLFTDFDSQINVPKTMESGTFITDKTVLDMKAMDSKSNGAIAWSNQTSFTCQDIFKETNATYPSSDVPCDATLTEKSFETDMNLNFQNLSVMGLRILLLKVAGFNLLMTLRLWSS

SEQ ID NO: 27 - protein, 305 aa, Artificial Sequence
  Synthetic
MGPGLLCWALLCLLGAGLVDAGVTQSPTHLIKTRGQQVTLRCSPKSGHDTVSWYQQALGQGPQFIFQYYEEEERQRGNFPDRFSGHQFPNYSSELNVNALLLGDSALYLCASSLGQTNYGYTFGSGTRLTVVEDLRNVTPPKVSLFEPSKAEIANKQKATLVCLARGFFPDHVELSWWVNGKEVHSGVSTDPQAYKESNYSYCLSSRLRVSATFWHNPRNHFRCQVQFHGLSEEDKWPEGSPKPVTQNISAEAWGRADCGITSASYQQGVLSATILYEILLGKATLYAVLVSTLVVMAMVKRKNS

SEQ ID NO: 28 - DNA, 387 bp, Artificial Sequence
  Synthetic
atgaggcaagtggcgagagtgatcgtgttcctgaccctgagtactttgagccttgctaagaccacccagcccatctccatggactcatatgaaggacaagaagtgaacataacctgtagccacaacaacattgctacaaatgattatatcacgtggtaccaacagtttcccagccaaggaccacgatttattattcaaggatacaagacaaaagttacaaacgaagtggcctccctgtttatccctgccgacagaaagtccagcactctgagcctgccccgggtttccctgagcgacactgctgtgtactactgcctcgtgggtgacatggaccaggcaggaactgctctgatctttgggaagggaaccaccttatcagtgagttcc

SEQ ID NO: 29 - DNA, 396 bp, Artificial Sequence
  Synthetic
  misc_feature (385)..(385): n is a, c, g, or t
atgggccccgggctcctctgctgggcactgctttgtctcctgggagcaggcttagtggacgctggagtcacccaaagtcccacacacctgatcaaaacgagaggacagcaagtgactctgagatgctctcctaagtctgggcatgacactgtgtcctggtaccaacaggccctgggtcaggggccccagtttatctttcagtattatgaggaggaagagagacagagaggcaacttccctgatcgattctcaggtcaccagttccctaactatagctctgagctgaatgtgaacgccttgttgctgggggactcggccctctatctctgtgccagcagcttgggacagaccaactatggctacaccttcggttcggggaccaggntaaccgttgta

SEQ ID NO: 30 - protein, 10 aa, Homo sapiens
GADGVGKSAL

SEQ ID NO: 31 - protein, 10 aa, Homo sapiens
VGADGVGKSA

SEQ ID NO: 32 - protein, 10 aa, Homo sapiens
VGAGGVGKSA

SEQ ID NO: 33 - protein, 10 aa, Homo sapiens
GAGGVGKSAL